European Patent Specification EP 3 347 044 B1, published April 19, 2023. Title: BIRD FLU VACCINE COMBINATION COMPRISING VIRUS-LIKE PARTICLES AND NOVEL ADJUVANTS. Applicant: ACADEMIA SINICA. The sequence listing filed with the application follows.

SEQUENCE LISTING (8 sequences)

SEQ ID NO: 1 - protein, 241 aa, Foot-and-mouth disease virus
MASMTGGQQMGRGSGIFPVACSDGYGGLVTTDPKTADPVYGKVFNPPRNLLPGRFTNLLDVAEACPTFLHFDGDVPYVTTKTDSDRVLAQFDLSLAAKHMSNTFLAGLAQYYTQYSGTINLHFMFTGPTDAKARYMVAYAPPGMEPPKTPEAAAHCIHAEWDTGLNSKFTFSIPYLSAADYAYTASDBAETTMBQGWBCLFQITHGKADGDALVVLASAGKDFDLRLPVDARTQLEHHHHH

SEQ ID NO: 2 - protein, 220 aa, Foot-and-mouth disease virus
GIFPVACSDGYGGLVTTDPKTADPVYGKVFNPPRNLLPGRFTNLLDVAEACPTFLHFDGDVPYVTTKTDSDRVLAQFDLSLAAKHMSNTFLAGLAQYYTQYSGTINLHFMFTGPTDAKARYMVAYAPPGMEPPKTPEAAAHCIHAEWDTGLNSKFTFSIPYLSAADYAYTASDBAETTMBQGWBCLFQITHGKADGDALVVLASAGKDFDLRLPVDARTQ

SEQ ID NO: 3 - protein, 60 aa, Foot-and-mouth disease virus
LAGLAQYYTQYSGTINLHFMFTGPTDAKARYMVAYAPPGMEPPKTPEAAAHCIHAEWDTG

SEQ ID NO: 4 - protein, 330 aa, Foot-and-mouth disease virus
HHHHHHMSDSEVNQEAKPEVKPEVKPETHINLKVSDGSSEIFFKIKKTTPLRRLMEAFAKRQGKEMDSLRFLYDGIRIQADQTPEDLDMEDNDIIEAHREQIGGATYGGMGIFPVACSDGYGGLVTTDPKTADPVYGKVFNPPRNLLPGRFTNLLDVAEACPTFLHFDGDVPYVTTKTDSDRVLAQFDLSLAAKHMSNTFLAGLAQYYTQYSGTINLHFMFTGPTDAKARYMVAYAPPGMEPPKTPEAAAHCIHAEWDTGLNSKFTFSIPYLSAADYAYTASDBAETTMBQGWBCLFQITHGKADGDALVVLASAGKDFDLRLPVDARTQ

SEQ ID NO: 5 - protein, 252 aa, Avian influenza virus
MSLLTEVETYVLSIVPSGPLKAEIAQRLEDVFAGKNTDLEALMEWLKTRPILSPLTKGILGFVFTLTVPSERGLQRRRFVQNALNGNGDPNNMDKAVKLYRKLKREITFHGAKEIALSYSAGALASCMGLIYNRMGAVTTEVAFGLVCATCEQIADSQHRSHRQMVATTNPLIRHENRMVLASTTAKAMEQMAGSSEQAAEAMEIASQARQMVQAMRAIGTHPSSSTGLRDDLLENLQTYQKRMGVQMQRFK

SEQ ID NO: 6 - protein, 97 aa, Avian influenza virus
MSLLTEVETPIRNEWGCRCNDSSDPLVVAANIIGILHLILWILDRLFFKCVYRLFKHGLKRGPSTEGVPESMREEYRKEQQNAVDADDSHFVSIELE

SEQ ID NO: 7 - protein, 564 aa, Avian influenza virus
MERIVIAFAIVNIVTGDRICIGYHANNSTTQVDTIMEKNVTVTHAQDILEKEHNGRLCSLKGVKPLILKNCSVAGWLLGNPMCDEFLNAPEWSYIVEKDRPSNGLCYPGTFNYYEELKHLMSSTNQFEKIQIFPRSSWSNHDASSGVSSACPYNGRSSFFRNVVWLIKKNNVYRTITRTYNNTNIEDLLIIWGIHHPNNAAEQIKLYQNPSTYVSVGTSTLNQRSIPEIATRPKVNGQSGRMEFFWTILRPNDSITFESTGNFIAPEYAYKIVKKGDSAIMKSELSYSNCDTKCQTPVGAINSSMPFHNVHPFAIGECPKYVKLKKLVLATGLRNIPQRRKRGLFGAIAGFIEGGWQGMVDGWYGYHHSNEQGSGYAADKESTQKAVDGITNKVNSIISKMNSQFEAVGKEFNNLERRIENLNKKMEDGFIDVWTYNAELLVLMENERTLDLHDSNVKNLYDKVRRQLRDNAKELGNGCFEFYHRCDNKCMESVRNGTYDYPQYSEESRLKREEIDGVKLESMGVYQIISIYSTVASSLALAIMVAGLSFWMCSNGSLQCRVCI

SEQ ID NO: 8 - protein, 449 aa, Avian influenza virus
MNPNQKIITIGSVSLTIATVCFLMQIAILTMTVTLHFNQNECSIPANNQVVPCEPIIIEKSINYRDWSKPQCRITGFAPFSKDNSIRLSAGGNIWVTREPYVSCDTSKCYQFALGQGTTLDNKHSNGTIHDRTPHRTLLMSELGVPFHLGTKQVCIAWSSSSCHDGKAWLHVCVTGDDKNATASFIYDGMLVDSIGSWSQNILRTQESECVCINGTCTVVMTDGSASGKADTRILFIEEGQVIHISPLSGSAQHIEECSCYPRYPNVRCVCRDNWKGSNRPVVDINMADYSIDSSYVCSGLVGDTPRNDDSSSSSNCRDPNNEKGNPGVKGWAFDDGDDIWMGRTISKDSRSGYETFRVIDGWTIANSKSQINRQVIVDNNNWSGYSGIFSVENKSCINRCFYVELIRGRPKETRVWWTSNSIVAFCGTSGTYGTGSWPDGANINFMPI